European Patent Application EP 4 628 500 A1, published October 8, 2025. Title: A novel Tellurium resistance membrane protein transporter variant and preparation method of L-amino acid using thereof. Applicant: CJ CheilJedang Corporation. The sequence listing filed with the application follows.

SEQUENCE LISTING (8 sequences)

SEQ ID NO: 1 - protein, 369 aa, unidentified
MEVNLATWLITIAVIAGFFIFDFYSHVRTPHEPTIKESAWWSLFYVGLACVFGIFLWFVWGEPGNPHQHGIEFFTGYVTEKALSVDNLFIFALIMGAFKIPRKYQQKVLLIGIALALVFRLVFILLGAAIIEAWSDVFYIFSIWLIYTAVKLLWDEVRDTPETDPNDMFIIKALRKVIPVTEGYHGDKLTHRFGGKLHLTPLFVALVSIGMVDLMFALDSIPAIYGITTEPYIVFTTNAFALLGLRQMYFLLDGLLDRLVYLPYGLGLILLFIGAKLGLHALHENNLPFINGGENVSVPEVSTVFSLVFIIGVLTITVIASIIKNKRDENQGGIPPKWNAAKYEGDNWETGEEPETGSATVTDISSEKK

SEQ ID NO: 2 - DNA, 1110 bp, unidentified
  source 1..1110: mol_type = genomic DNA
atggaagtaaacttagccacatggctaatcactatcgcagtgattgctggcttcttcattttcgatttctattcccacgtccgcaccccacacgagcccaccattaaagaatccgcatggtggagcttgttctatgtcggtcttgcctgtgtattcggcatcttcttgtggttcgtttggggcgagcctggtaacccacaccagcacggcatcgagttcttcacgggttacgtcacagagaaggcactgagcgttgataacttgtttatcttcgcgctgatcatgggtgcctttaagattccgcgtaagtaccagcaaaaggtactcctcatcggtattgcactggctctggtcttccgcctcgtgttcatcctcctcggcgctgcaattatcgaagcatggtccgatgtcttctacatcttctccatctggctgatctacaccgctgtgaagctcctgtgggacgaagttcgagacacccctgagaccgacccgaacgacatgttcatcattaaggcgctgcgcaaggtcattccggttactgagggctaccacggcgacaagctcactcaccgcttcggaggcaagctgcacctgaccccactgtttgttgctcttgtatccatcggcatggttgacctgatgttcgcactggactctatcccagcgatttacggcatcaccacggagccttacatcgtgttcaccactaacgcattcgccctgctgggtctgcgccaaatgtacttcctgcttgatggtctgctagaccgcctggtctacctgccttatggcttgggtcttatcctgctgttcattggtgcaaagcttggtctgcatgcactgcacgaaaacaacctgccattcatcaacggtggtgaaaacgtctccgtacctgaggtttccaccgtattctccttggtcttcatcattggtgtcctgacaatcaccgtcatcgcatccatcatcaagaacaaacgcgacgaaaaccagggcggtattccaccaaagtggaacgctgcaaagtatgagggcgacaactgggagaccggtgaggagcctgaaaccggatccgccaccgttaccgatatctcctcagagaagaagtaa

SEQ ID NO: 3 - protein, 369 aa, synthetic construct
MEVNLATWLITIAVIAGFFIFDFYSHVRTPHEPTIKESAWWSLFYVGLACVFGIFLWFVWGEPGNPHQHGIEFFTGYVTEKALSVDNLFIFALIMGAFKIPRKYQQKVLLIGIALALVFRLVFILLGAAIIEAWSDVFYIFSIWLIYTAVKLLWDEVRDTPETDPNDMFIIKALRKVIPVTEGYHGDKLTHRFGGKLHLTPLFVALVSIGMVDLMFALDSIPAIYGITTESYIVFTTNAFALLGLRQMYFLLDGLLDRLVYLPYGLGLILLFIGAKLGLHALHENNLPFINGGENVSVPEVSTVFSLVFIIGVLTITVIASIIKNKRDENQGGIPPKWNAAKYEGDNWETGEEPETGSATVTDISSEKK

SEQ ID NO: 4 - DNA, 1110 bp, synthetic construct
  source 1..1110: mol_type = other DNA
atggaagtaaacttagccacatggctaatcactatcgcagtgattgctggcttcttcattttcgatttctattcccacgtccgcaccccacacgagcccaccattaaagaatccgcatggtggagcttgttctatgtcggtcttgcctgtgtattcggcatcttcttgtggttcgtttggggcgagcctggtaacccacaccagcacggcatcgagttcttcacgggttacgtcacagagaaggcactgagcgttgataacttgtttatcttcgcgctgatcatgggtgcctttaagattccgcgtaagtaccagcaaaaggtactcctcatcggtattgcactggctctggtcttccgcctcgtgttcatcctcctcggcgctgcaattatcgaagcatggtccgatgtcttctacatcttctccatctggctgatctacaccgctgtgaagctcctgtgggacgaagttcgagacacccctgagaccgacccgaacgacatgttcatcattaaggcgctgcgcaaggtcattccggttactgagggctaccacggcgacaagctcactcaccgcttcggaggcaagctgcacctgaccccactgtttgttgctcttgtatccatcggcatggttgacctgatgttcgcactggactctatcccagcgatttacggcatcaccacggagtcttacatcgtgttcaccactaacgcattcgccctgctgggtctgcgccaaatgtacttcctgcttgatggtctgctagaccgcctggtctacctgccttatggcttgggtcttatcctgctgttcattggtgcaaagcttggtctgcatgcactgcacgaaaacaacctgccattcatcaacggtggtgaaaacgtctccgtacctgaggtttccaccgtattctccttggtcttcatcattggtgtcctgacaatcaccgtcatcgcatccatcatcaagaacaaacgcgacgaaaaccagggcggtattccaccaaagtggaacgctgcaaagtatgagggcgacaactgggagaccggtgaggagcctgaaaccggatccgccaccgttaccgatatctcctcagagaagaagtaa

SEQ ID NO: 5 - DNA, 34 bp, synthetic construct
  source 1..34: mol_type = other DNA
cggtacccggggatccgtaacccacaccagcacg

SEQ ID NO: 6 - DNA, 32 bp, synthetic construct
  source 1..32: mol_type = other DNA
aacacgatgtaagactccgtggtgatgccgta

SEQ ID NO: 7 - DNA, 35 bp, synthetic construct
  source 1..35: mol_type = other DNA
tcaccacggagtcttacatcgtgttcaccactaac

SEQ ID NO: 8 - DNA, 34 bp, synthetic construct
  source 1..34: mol_type = other DNA
atgcctgcaggtcgacgttgctgcctaaaccagc